European Patent Application EP 4 620 972 A1, published September 24, 2025. Title: Dual gene-engineered immune cell using CTLA4 mutant and chimeric antigen receptor and use thereof. Applicant: Seoul National University R&DB Foundation. The sequence listing filed with the application follows.

SEQUENCE LISTING (23 sequences)

SEQ ID NO: 1 - protein, 223 aa, synthetic construct
MACLGFQRHKAQLNLATRTWPCTLLFFLLFIPVFCKAMHVAQPAVVLASSRGIASFVCEYASPGKATEVRVTVLRQADSQVTEVCAATYMMGNELTFLDDSICTGTSSGNQVNLTIQGLRAMDTGLYICKVELMYPPPYYLGIGNGTQIYVIDPEPCPDSDFLLWILAAVSSGLFFYSFLLTAVSLSKMLKKRSPLTTGVYVKMPPTEPECEKQFQPYFIPIN

SEQ ID NO: 2 - protein, 223 aa, synthetic construct
MACLGLRRYKAQLQLPSRTWPFVALLTLLFIPVFSEAIQVTQPSVVLASSHGVASFPCEYSPSHNTDEVRVTVLRQTNDQMTEVCATTFTEKNTVGFLDYPFCSGTFNESRVNLTIQGLRAVDTGLYLCKVELMYPPPYFVGMGNGTQIYVIDPEPCPDSDFLLWILVAVSLGLFFYSFLVTAVSLSKMLKKRSPLTTGVYVKMPPTEPECEKQFQPYFIPIN

SEQ ID NO: 3 - protein, 220 aa, synthetic construct
MLRLLLALNLFPSIQVTGNKILVKQSPMLVAYDNAVNLSCKYSYNLFSREFRASLHKGLDSAVEVCVVYGNYSQQLQVYSKTGFNCDGKLGNESVTFYLQNLYVNQTDIYFCKIEVMYPPPYLDNEKSNGTIIHVKGKHLCPSPLFPGPSKPFWVLVVVGGVLACYSLLVTVAFIIFWVRSKRSRLLHSDYMNMTPRRPGPTRKHYQPYAPPRDFAAYRS

SEQ ID NO: 4 - protein, 218 aa, synthetic construct
MTLRLLFLALNFFSVQVTENKILVKQSPLLVVDSNEVSLSCRYSYNLLAKEFRASLYKGVNSDVEVCVGNGNFTYQPQFRSNAEFNCDGDFDNETVTFRLWNLHVNHTDIYFCKIEFMYPPPYLDNERSNGTIIHIKEKHLCHTQSSPKLFWALVVVAGVLFCYGLLVTVALCVIWTNSRRNRLLQSDYMNMTPRRPGLTRKPYQPYAPARDFAAYRP

SEQ ID NO: 5 - protein, 231 aa, synthetic construct
MACLGFQRHKAQLNLATRTWPCTLLFFLLFIPVFCKAMHVAQPAVVLASSRGIASFVCEYASPGKATEVRVTVLRQADSQVTEVCAATYMMGNELTFLDDSICTGTSSGNQVNLTIQGLRAMDTGLYICKVELMYPPPYYLGIGNGTQIYVIDPEPCPDSDFLLWILAAVSSGLFFYSFLLTAVSLSKMVRSKRSRLLHSDYMNMTPRRPGPTRKHYQPYAPPRDFAAYRS

SEQ ID NO: 6 - protein, 231 aa, synthetic construct
MACLGLRRYKAQLQLPSRTWPFVALLTLLFIPVFSEAIQVTQPSVVLASSHGVASFPCEYSPSHNTDEVRVTVLRQTNDQMTEVCATTFTEKNTVGFLDYPFCSGTFNESRVNLTIQGLRAVDTGLYLCKVELMYPPPYFVGMGNGTQIYVIDPEPCPDSDFLLWILVAVSLGLFFYSFLVTAVSLSKMTNSRRNRLLQSDYMNMTPRRPGLTRKPYQPYAPARDFAAYRP

SEQ ID NO: 7 - protein, 229 aa, synthetic construct
MACLGFQRHKAQLNLATRTWPCTLLFFLLFIPVFCKAMHVAQPAVVLASSRGIASFVCEYASPGKATEVRVTVLRQADSQVTEVCAATYMMGNELTFLDDSICTGTSSGNQVNLTIQGLRAMDTGLYICKVELMYPPPYYLGIGNGTQIYVIDPEPCPDSDFWVLVVVGGVLACYSLLVTVAFIIFWVRSKRSRLLHSDYMNMTPRRPGPTRKHYQPYAPPRDFAAYRS

SEQ ID NO: 8 - DNA, 1338 bp, synthetic construct
  source 1..1338: mol_type = other DNA
atggcctcaccgttgacccgctttctgtcgctgaacctgctgctgctgggtgagtcgattatcctggggagtggagaagctgacatccagatgacccagagccctgccagcctgtctaccagcctgggcgagacagtgaccatccagtgtcaggccagcgaggacatctactctggcctggcttggtatcagcagaagcccggcaagagccctcagctgctgatctacggcgccagcgacctgcaggacggcgtgcctagcagattcagcggcagcggctccggaacccagtacagcctgaagatcaccagcatgcagaccgaggacgagggcgtgtacttctgccagcaaggcctgacctaccctagaaccttcggaggaggcaccaagctggaactgaagggcggaggcggaagtggaggcggaggatctggcggcggaggctctgaagtgcagctgcagcagtctggcgctgaactggtccggcctggcactagcgtgaagctgtcctgcaaggtgtccggcgacaccatcaccttctactacatgcacttcgtgaagcagaggccaggacagggcctggaatggatcggcagaatcgaccctgaggacgagagcaccaagtacagcgagaagttcaagaacaaggccaccctgaccgccgacaccagcagcaacaccgcctacctgaagctgtctagcctgacctccgaggacaccgccacctacttttgcatctacggcggctactacttcgactactggggccagggcgtgatggtcaccgtgtccagcactactaccaagccagtgctgcgaactccctcacctgtgcaccctaccgggacatctcagccccagagaccagaagattgtcggccccgtggctcagtgaaggggaccggattggacttcgcctgtgatatttacatctgggcacccttggccggaatctgcgtggcccttctgctgtccttgatcatcactctcatctgcagagcaaaattcagcaggagtgcagagactgctgccaacctgcaggaccccaaccagctctacaatgagctcaatctagggcgaagagaggaatatgacgtcttggagaagaagcgggctcgggatccagagatgggaggcaaacagcagaggaggaggaacccccaggaaggcgtatacaatgcactgcagaaagacaagatggcagaagcctacagtgagatcggcacaaaaggcgagaggcggagaggcaaggggcacgatggcctttaccagggtctcagcactgccaccaaggacacctatgatgccctgcatatgcagaccctggcccctcgctaa

SEQ ID NO: 9 - protein, 445 aa, synthetic construct
MASPLTRFLSLNLLLLGESIILGSGEADIQMTQSPASLSTSLGETVTIQCQASEDIYSGLAWYQQKPGKSPQLLIYGASDLQDGVPSRFSGSGSGTQYSLKITSMQTEDEGVYFCQQGLTYPRTFGGGTKLELKGGGGSGGGGSGGGGSEVQLQQSGAELVRPGTSVKLSCKVSGDTITFYYMHFVKQRPGQGLEWIGRIDPEDESTKYSEKFKNKATLTADTSSNTAYLKLSSLTSEDTATYFCIYGGYYFDYWGQGVMVTVSSTTTKPVLRTPSPVHPTGTSQPQRPEDCRPRGSVKGTGLDFACDIYIWAPLAGICVALLLSLIITLICRAKFSRSAETAANLQDPNQLYNELNLGRREEYDVLEKKRARDPEMGGKQQRRRNPQEGVYNALQKDKMAEAYSEIGTKGERRRGKGHDGLYQGLSTATKDTYDALHMQTLAPR

SEQ ID NO: 10 - DNA, 1428 bp, synthetic construct
  source 1..1428: mol_type = other DNA
atgggtgtccctacccagctcctgggactgctcctgctgtggatcaccgacgccatctgcgacatccagatgacccagagccctgccagcctgtctaccagcctgggcgagacagtgaccatccagtgtcaggccagcgaggacatctactctggcctggcttggtatcagcagaagcccggcaagagccctcagctgctgatctacggcgccagcgacctgcaggacggcgtgcctagcagattcagcggcagcggctccggaacccagtacagcctgaagatcaccagcatgcagaccgaggacgagggcgtgtacttctgccagcaaggcctgacctaccctagaaccttcggaggaggcaccaagctggaactgaagggcggaggcggaagtggaggcggaggatctggcggcggaggctctgaagtgcagctgcagcagtctggcgctgaactggtccggcctggcactagcgtgaagctgtcctgcaaggtgtccggcgacaccatcaccttctactacatgcacttcgtgaagcagaggccaggacagggcctggaatggatcggcagaatcgaccctgaggacgagagcaccaagtacagcgagaagttcaagaacaaggccaccctgaccgccgacaccagcagcaacaccgcctacctgaagctgtctagcctgacctccgaggacaccgccacctacttttgcatctacggcggctactacttcgactactggggccagggcgtgatggtcaccgtgtccagcatcgagttcatgtacccccctccctacctggacaacgagagaagcaacggcaccatcatccacatcaaagaaaagcacctgtgccacacccagagcagccccaagctgttctgggccctggtggtggtggccggcgtgctgttctgttacggcctgctggtcacagtggccctgtgcgtgatctggaccaacagcagaagaaacagaggcggccagagcgactacatgaacatgacccccagaaggccaggcctgaccagaaagccctaccagccctacgcccctgccagagacttcgccgcctacagacccagagccaagttcagcagatccgccgagacagccgccaacctgcaggatcccaaccagctgttcaacgagctgaacctgggcagacgggaggaattcgacgtgctggaaaagaagagagccagggaccccgagatgggcggcaagcagcagagaagaagaaaccctcaggaaggcgtctacaacgccctgcagaaagacaagatggccgaggcctacagcgagatcggcaccaagggcgagagaagaaggggcaagggccacgatggcctgttccagggcctgtccaccgccaccaaggacaccttcgacgccctgcacatgcagaccctggcccccagatga

SEQ ID NO: 11 - protein, 475 aa, synthetic construct
MGVPTQLLGLLLLWITDAICDIQMTQSPASLSTSLGETVTIQCQASEDIYSGLAWYQQKPGKSPQLLIYGASDLQDGVPSRFSGSGSGTQYSLKITSMQTEDEGVYFCQQGLTYPRTFGGGTKLELKGGGGSGGGGSGGGGSEVQLQQSGAELVRPGTSVKLSCKVSGDTITFYYMHFVKQRPGQGLEWIGRIDPEDESTKYSEKFKNKATLTADTSSNTAYLKLSSLTSEDTATYFCIYGGYYFDYWGQGVMVTVSSIEFMYPPPYLDNERSNGTIIHIKEKHLCHTQSSPKLFWALVVVAGVLFCYGLLVTVALCVIWTNSRRNRGGQSDYMNMTPRRPGLTRKPYQPYAPARDFAAYRPRAKFSRSAETAANLQDPNQLFNELNLGRREEFDVLEKKRARDPEMGGKQQRRRNPQEGVYNALQKDKMAEAYSEIGTKGERRRGKGHDGLFQGLSTATKDTFDALHMQTLAPR

SEQ ID NO: 12 - DNA, 1464 bp, synthetic construct
  source 1..1464: mol_type = other DNA
atggcctcaccgttgacccgctttctgtcgctgaacctgctgctgctgggtgagtcgattatcctggggagtggagaagctgacatccagatgacccagagccctgccagcctgtctaccagcctgggcgagacagtgaccatccagtgtcaggccagcgaggacatctactctggcctggcttggtatcagcagaagcccggcaagagccctcagctgctgatctacggcgccagcgacctgcaggacggcgtgcctagcagattcagcggcagcggctccggaacccagtacagcctgaagatcaccagcatgcagaccgaggacgagggcgtgtacttctgccagcaaggcctgacctaccctagaaccttcggaggaggcaccaagctggaactgaagggcggaggcggaagtggaggcggaggatctggcggcggaggctctgaagtgcagctgcagcagtctggcgctgaactggtccggcctggcactagcgtgaagctgtcctgcaaggtgtccggcgacaccatcaccttctactacatgcacttcgtgaagcagaggccaggacagggcctggaatggatcggcagaatcgaccctgaggacgagagcaccaagtacagcgagaagttcaagaacaaggccaccctgaccgccgacaccagcagcaacaccgcctacctgaagctgtctagcctgacctccgaggacaccgccacctacttttgcatctacggcggctactacttcgactactggggccagggcgtgatggtcaccgtgtccagcactactaccaagccagtgctgcgaactccctcacctgtgcaccctaccgggacatctcagccccagagaccagaagattgtcggccccgtggctcagtgaaggggaccggattggacttcgcctgtgatatttacatctgggcacccttggccggaatctgcgtggcccttctgctgtccttgatcatcactctcatctgcaaacggggcagaaagaaactcctgtatatattcaaacaaccatttatgagaccagtacaaactactcaagaggaagatggctgtagctgccgatttccagaagaagaagaaggaggatgtgaactgagagcaaaattcagcaggagtgcagagactgctgccaacctgcaggaccccaaccagctctacaatgagctcaatctagggcgaagagaggaatatgacgtcttggagaagaagcgggctcgggatccagagatgggaggcaaacagcagaggaggaggaacccccaggaaggcgtatacaatgcactgcagaaagacaagatggcagaagcctacagtgagatcggcacaaaaggcgagaggcggagaggcaaggggcacgatggcctttaccagggtctcagcactgccaccaaggacacctatgatgccctgcatatgcagaccctggcccctcgctaa

SEQ ID NO: 13 - protein, 487 aa, synthetic construct
MASPLTRFLSLNLLLLGESIILGSGEADIQMTQSPASLSTSLGETVTIQCQASEDIYSGLAWYQQKPGKSPQLLIYGASDLQDGVPSRFSGSGSGTQYSLKITSMQTEDEGVYFCQQGLTYPRTFGGGTKLELKGGGGSGGGGSGGGGSEVQLQQSGAELVRPGTSVKLSCKVSGDTITFYYMHFVKQRPGQGLEWIGRIDPEDESTKYSEKFKNKATLTADTSSNTAYLKLSSLTSEDTATYFCIYGGYYFDYWGQGVMVTVSSTTTKPVLRTPSPVHPTGTSQPQRPEDCRPRGSVKGTGLDFACDIYIWAPLAGICVALLLSLIITLICKRGRKKLLYIFKQPFMRPVQTTQEEDGCSCRFPEEEEGGCELRAKFSRSAETAANLQDPNQLYNELNLGRREEYDVLEKKRARDPEMGGKQQRRRNPQEGVYNALQKDKMAEAYSEIGTKGERRRGKGHDGLYQGLSTATKDTYDALHMQTLAPR

SEQ ID NO: 14 - DNA, 1448 bp, synthetic construct
  source 1..1448: mol_type = other DNA
atggccttaccagtgaccgccttgctcctgccgctggccttgctgctccacgccgccaggccggacatccagatgacacagactacatcctccctgtctgcctctctgggagacagagtcaccatcagttgcagggcaagtcaggacattagtaaatatttaaattggtatcagcagaaaccagatggaactgttaaactcctgatctaccatacatcaagattacactcaggagtcccatcaaggttcagtggcagtgggtctggaacagattattctctcaccattagcaacctggagcaagaagatattgccacttacttttgccaacagggtaatacgcttccgtacacgttcggaggggggaccaagctggagatcacaggtggcggtggctcgggcggtggtgggtcgggtggcggcggatctgaggtgaaactgcaggagtcaggacctggcctggtggcgccctcacagagcctgtccgtcacatgcactgtctcaggggtctcattacccgactatggtgtaagctggattcgccagcctccacgaaagggtctggagtggctgggagtaatatggggtagtgaaaccacatactataattcagctctcaaatccagactgaccatcatcaaggacaactccaagagccaagttttcttaaaaatgaacagtctgcaaactgatgacacagccatttactactgtgccaaacattattactacggtggtagctatgctatggactactggggccaaggaacctcagtcaccgtctcctcaaccacgacgccagcgccgcgaccaccaacaccggcgcccaccatcgcgtcgcagcccctgtccctgcgcccagaggcgtgccggccagcggcggggggcgcagtgcacacgagggggctggacttcgcctgtgatatctacatctgggcgcccttggccgggacttgtggggtccttctcctgtcactggttatcaccctttactgcaaacggggcagaaagaaactcctgtatatattcaaacaaccatttatgagaccagtacaaactactcaagaggaagatggctgtagctgccgatttccagaagaagaagaaggaggatgtgaactgagagtgaagttcagcaggagcgcagacgcccccgcgtacaagcagggccagaaccagctctataacgagctcaatctaggacgaagagaggagtacgatgttttggacaagagacgtggccgggaccctgagatggggggaaagccgagaaggaagaaccctcaggaaggcctgtacaatgaactgcagaaagataagatggcggaggcctacagtgagattgggatgaaaggcgagcgccggaggggcaaggggcacgatggcctttaccagggtctcagtacagccaccaaggacacctacgacgcccttcacatgcaggccct

SEQ ID NO: 15 - protein, 486 aa, synthetic construct
MALPVTALLLPLALLLHAARPDIQMTQTTSSLSASLGDRVTISCRASQDISKYLNWYQQKPDGTVKLLIYHTSRLHSGVPSRFSGSGSGTDYSLTISNLEQEDIATYFCQQGNTLPYTFGGGTKLEITGGGGSGGGGSGGGGSEVKLQESGPGLVAPSQSLSVTCTVSGVSLPDYGVSWIRQPPRKGLEWLGVIWGSETTYYNSALKSRLTIIKDNSKSQVFLKMNSLQTDDTAIYYCAKHYYYGGSYAMDYWGQGTSVTVSSTTTPAPRPPTPAPTIASQPLSLRPEACRPAAGGAVHTRGLDFACDIYIWAPLAGTCGVLLLSLVITLYCKRGRKKLLYIFKQPFMRPVQTTQEEDGCSCRFPEEEEGGCELRVKFSRSADAPAYKQGQNQLYNELNLGRREEYDVLDKRRGRDPEMGGKPRRKNPQEGLYNELQKDKMAEAYSEIGMKGERRRGKGHDGLYQGLSTATKDTYDALHMQALPPR

SEQ ID NO: 16 - DNA, 2097 bp, synthetic construct
  source 1..2097: mol_type = other DNA
atggcctcaccgttgacccgctttctgtcgctgaacctgctgctgctgggtgagtcgattatcctggggagtggagaagctgacatccagatgacccagagccctgccagcctgtctaccagcctgggcgagacagtgaccatccagtgtcaggccagcgaggacatctactctggcctggcttggtatcagcagaagcccggcaagagccctcagctgctgatctacggcgccagcgacctgcaggacggcgtgcctagcagattcagcggcagcggctccggaacccagtacagcctgaagatcaccagcatgcagaccgaggacgagggcgtgtacttctgccagcaaggcctgacctaccctagaaccttcggaggaggcaccaagctggaactgaagggcggaggcggaagtggaggcggaggatctggcggcggaggctctgaagtgcagctgcagcagtctggcgctgaactggtccggcctggcactagcgtgaagctgtcctgcaaggtgtccggcgacaccatcaccttctactacatgcacttcgtgaagcagaggccaggacagggcctggaatggatcggcagaatcgaccctgaggacgagagcaccaagtacagcgagaagttcaagaacaaggccaccctgaccgccgacaccagcagcaacaccgcctacctgaagctgtctagcctgacctccgaggacaccgccacctacttttgcatctacggcggctactacttcgactactggggccagggcgtgatggtcaccgtgtccagcactactaccaagccagtgctgcgaactccctcacctgtgcaccctaccgggacatctcagccccagagaccagaagattgtcggccccgtggctcagtgaaggggaccggattggacttcgcctgtgatatttacatctgggcacccttggccggaatctgcgtggcccttctgctgtccttgatcatcactctcatctgcagagcaaaattcagcaggagtgcagagactgctgccaacctgcaggaccccaaccagctctacaatgagctcaatctagggcgaagagaggaatatgacgtcttggagaagaagcgggctcgggatccagagatgggaggcaaacagcagaggaggaggaacccccaggaaggcgtatacaatgcactgcagaaagacaagatggcagaagcctacagtgagatcggcacaaaaggcgagaggcggagaggcaaggggcacgatggcctttaccagggtctcagcactgccaccaaggacacctatgatgccctgcatatgcagaccctggcccctcgcggaagcggagctactaacttcagcctgctgaagcaggctggagacgtggaggagaaccctggacctatggcttgtcttggactccggaggtacaaagctcaactgcagctgccttctaggacttggccttttgtagccctgctcactcttcttttcatcccagtcttctctgaagccatacaggtgacccaaccttcagtggtgttggctagcagccatggtgtcgccagctttccatgtgaatattcaccgtcacacaacactgatgaggtccgggtgactgtgctgcggcagacaaatgaccaaatgactgaggtctgtgccacgacattcacagagaagaatacagtgggcttcctagattaccccttctgcagtggtacctttaatgaaagcagagtgaacctcaccatccaaggactgagagctgttgacacgggactgtacctctgcaaggtggaactcatgtacccaccgccatactttgtgggcatgggcaacgggacgcagatttatgtcattgatccagaaccatgcccggattctgacttcctcctttggatccttgtcgcagttagcttggggttgtttttttacagtttcctggtcactgctgtttctttgagcaagatgacaaatagtagaaggaacagactccttcaaagtgactacatgaacatgactccccggaggcctgggctcactcgaaagccttaccagccctacgcccctgccagagactttgcagcgtaccgcccctga

SEQ ID NO: 17 - protein, 698 aa, synthetic construct
MASPLTRFLSLNLLLLGESIILGSGEADIQMTQSPASLSTSLGETVTIQCQASEDIYSGLAWYQQKPGKSPQLLIYGASDLQDGVPSRFSGSGSGTQYSLKITSMQTEDEGVYFCQQGLTYPRTFGGGTKLELKGGGGSGGGGSGGGGSEVQLQQSGAELVRPGTSVKLSCKVSGDTITFYYMHFVKQRPGQGLEWIGRIDPEDESTKYSEKFKNKATLTADTSSNTAYLKLSSLTSEDTATYFCIYGGYYFDYWGQGVMVTVSSTTTKPVLRTPSPVHPTGTSQPQRPEDCRPRGSVKGTGLDFACDIYIWAPLAGICVALLLSLIITLICRAKFSRSAETAANLQDPNQLYNELNLGRREEYDVLEKKRARDPEMGGKQQRRRNPQEGVYNALQKDKMAEAYSEIGTKGERRRGKGHDGLYQGLSTATKDTYDALHMQTLAPRGSGATNFSLLKQAGDVEENPGPMACLGLRRYKAQLQLPSRTWPFVALLTLLFIPVFSEAIQVTQPSVVLASSHGVASFPCEYSPSHNTDEVRVTVLRQTNDQMTEVCATTFTEKNTVGFLDYPFCSGTFNESRVNLTIQGLRAVDTGLYLCKVELMYPPPYFVGMGNGTQIYVIDPEPCPDSDFLLWILVAVSLGLFFYSFLVTAVSLSKMTNSRRNRLLQSDYMNMTPRRPGLTRKPYQPYAPARDFAAYRP

SEQ ID NO: 18 - DNA, 2187 bp, synthetic construct
  source 1..2187: mol_type = other DNA
atgggtgtccctacccagctcctgggactgctcctgctgtggatcaccgacgccatctgcgacatccagatgacccagagccctgccagcctgtctaccagcctgggcgagacagtgaccatccagtgtcaggccagcgaggacatctactctggcctggcttggtatcagcagaagcccggcaagagccctcagctgctgatctacggcgccagcgacctgcaggacggcgtgcctagcagattcagcggcagcggctccggaacccagtacagcctgaagatcaccagcatgcagaccgaggacgagggcgtgtacttctgccagcaaggcctgacctaccctagaaccttcggaggaggcaccaagctggaactgaagggcggaggcggaagtggaggcggaggatctggcggcggaggctctgaagtgcagctgcagcagtctggcgctgaactggtccggcctggcactagcgtgaagctgtcctgcaaggtgtccggcgacaccatcaccttctactacatgcacttcgtgaagcagaggccaggacagggcctggaatggatcggcagaatcgaccctgaggacgagagcaccaagtacagcgagaagttcaagaacaaggccaccctgaccgccgacaccagcagcaacaccgcctacctgaagctgtctagcctgacctccgaggacaccgccacctacttttgcatctacggcggctactacttcgactactggggccagggcgtgatggtcaccgtgtccagcatcgagttcatgtacccccctccctacctggacaacgagagaagcaacggcaccatcatccacatcaaagaaaagcacctgtgccacacccagagcagccccaagctgttctgggccctggtggtggtggccggcgtgctgttctgttacggcctgctggtcacagtggccctgtgcgtgatctggaccaacagcagaagaaacagaggcggccagagcgactacatgaacatgacccccagaaggccaggcctgaccagaaagccctaccagccctacgcccctgccagagacttcgccgcctacagacccagagccaagttcagcagatccgccgagacagccgccaacctgcaggatcccaaccagctgttcaacgagctgaacctgggcagacgggaggaattcgacgtgctggaaaagaagagagccagggaccccgagatgggcggcaagcagcagagaagaagaaaccctcaggaaggcgtctacaacgccctgcagaaagacaagatggccgaggcctacagcgagatcggcaccaagggcgagagaagaaggggcaagggccacgatggcctgttccagggcctgtccaccgccaccaaggacaccttcgacgccctgcacatgcagaccctggcccccagaggaagcggagctactaacttcagcctgctgaagcaggctggagacgtggaggagaaccctggacctatggcttgtcttggactccggaggtacaaagctcaactgcagctgccttctaggacttggccttttgtagccctgctcactcttcttttcatcccagtcttctctgaagccatacaggtgacccaaccttcagtggtgttggctagcagccatggtgtcgccagctttccatgtgaatattcaccgtcacacaacactgatgaggtccgggtgactgtgctgcggcagacaaatgaccaaatgactgaggtctgtgccacgacattcacagagaagaatacagtgggcttcctagattaccccttctgcagtggtacctttaatgaaagcagagtgaacctcaccatccaaggactgagagctgttgacacgggactgtacctctgcaaggtggaactcatgtacccaccgccatactttgtgggcatgggcaacgggacgcagatttatgtcattgatccagaaccatgcccggattctgacttcctcctttggatccttgtcgcagttagcttggggttgtttttttacagtttcctggtcactgctgtttctttgagcaagatgacaaatagtagaaggaacagactccttcaaagtgactacatgaacatgactccccggaggcctgggctcactcgaaagccttaccagccctacgcccctgccagagactttgcagcgtaccgcccctga

SEQ ID NO: 19 - protein, 728 aa, synthetic construct
MGVPTQLLGLLLLWITDAICDIQMTQSPASLSTSLGETVTIQCQASEDIYSGLAWYQQKPGKSPQLLIYGASDLQDGVPSRFSGSGSGTQYSLKITSMQTEDEGVYFCQQGLTYPRTFGGGTKLELKGGGGSGGGGSGGGGSEVQLQQSGAELVRPGTSVKLSCKVSGDTITFYYMHFVKQRPGQGLEWIGRIDPEDESTKYSEKFKNKATLTADTSSNTAYLKLSSLTSEDTATYFCIYGGYYFDYWGQGVMVTVSSIEFMYPPPYLDNERSNGTIIHIKEKHLCHTQSSPKLFWALVVVAGVLFCYGLLVTVALCVIWTNSRRNRGGQSDYMNMTPRRPGLTRKPYQPYAPARDFAAYRPRAKFSRSAETAANLQDPNQLFNELNLGRREEFDVLEKKRARDPEMGGKQQRRRNPQEGVYNALQKDKMAEAYSEIGTKGERRRGKGHDGLFQGLSTATKDTFDALHMQTLAPRGSGATNFSLLKQAGDVEENPGPMACLGLRRYKAQLQLPSRTWPFVALLTLLFIPVFSEAIQVTQPSVVLASSHGVASFPCEYSPSHNTDEVRVTVLRQTNDQMTEVCATTFTEKNTVGFLDYPFCSGTFNESRVNLTIQGLRAVDTGLYLCKVELMYPPPYFVGMGNGTQIYVIDPEPCPDSDFLLWILVAVSLGLFFYSFLVTAVSLSKMTNSRRNRLLQSDYMNMTPRRPGLTRKPYQPYAPARDFAAYRP

SEQ ID NO: 20 - DNA, 2223 bp, synthetic construct
  source 1..2223: mol_type = other DNA
atggcctcaccgttgacccgctttctgtcgctgaacctgctgctgctgggtgagtcgattatcctggggagtggagaagctgacatccagatgacccagagccctgccagcctgtctaccagcctgggcgagacagtgaccatccagtgtcaggccagcgaggacatctactctggcctggcttggtatcagcagaagcccggcaagagccctcagctgctgatctacggcgccagcgacctgcaggacggcgtgcctagcagattcagcggcagcggctccggaacccagtacagcctgaagatcaccagcatgcagaccgaggacgagggcgtgtacttctgccagcaaggcctgacctaccctagaaccttcggaggaggcaccaagctggaactgaagggcggaggcggaagtggaggcggaggatctggcggcggaggctctgaagtgcagctgcagcagtctggcgctgaactggtccggcctggcactagcgtgaagctgtcctgcaaggtgtccggcgacaccatcaccttctactacatgcacttcgtgaagcagaggccaggacagggcctggaatggatcggcagaatcgaccctgaggacgagagcaccaagtacagcgagaagttcaagaacaaggccaccctgaccgccgacaccagcagcaacaccgcctacctgaagctgtctagcctgacctccgaggacaccgccacctacttttgcatctacggcggctactacttcgactactggggccagggcgtgatggtcaccgtgtccagcactactaccaagccagtgctgcgaactccctcacctgtgcaccctaccgggacatctcagccccagagaccagaagattgtcggccccgtggctcagtgaaggggaccggattggacttcgcctgtgatatttacatctgggcacccttggccggaatctgcgtggcccttctgctgtccttgatcatcactctcatctgcaaacggggcagaaagaaactcctgtatatattcaaacaaccatttatgagaccagtacaaactactcaagaggaagatggctgtagctgccgatttccagaagaagaagaaggaggatgtgaactgagagcaaaattcagcaggagtgcagagactgctgccaacctgcaggaccccaaccagctctacaatgagctcaatctagggcgaagagaggaatatgacgtcttggagaagaagcgggctcgggatccagagatgggaggcaaacagcagaggaggaggaacccccaggaaggcgtatacaatgcactgcagaaagacaagatggcagaagcctacagtgagatcggcacaaaaggcgagaggcggagaggcaaggggcacgatggcctttaccagggtctcagcactgccaccaaggacacctatgatgccctgcatatgcagaccctggcccctcgcggaagcggagctactaacttcagcctgctgaagcaggctggagacgtggaggagaaccctggacctatggcttgtcttggactccggaggtacaaagctcaactgcagctgccttctaggacttggccttttgtagccctgctcactcttcttttcatcccagtcttctctgaagccatacaggtgacccaaccttcagtggtgttggctagcagccatggtgtcgccagctttccatgtgaatattcaccgtcacacaacactgatgaggtccgggtgactgtgctgcggcagacaaatgaccaaatgactgaggtctgtgccacgacattcacagagaagaatacagtgggcttcctagattaccccttctgcagtggtacctttaatgaaagcagagtgaacctcaccatccaaggactgagagctgttgacacgggactgtacctctgcaaggtggaactcatgtacccaccgccatactttgtgggcatgggcaacgggacgcagatttatgtcattgatccagaaccatgcccggattctgacttcctcctttggatccttgtcgcagttagcttggggttgtttttttacagtttcctggtcactgctgtttctttgagcaagatgacaaatagtagaaggaacagactccttcaaagtgactacatgaacatgactccccggaggcctgggctcactcgaaagccttaccagccctacgcccctgccagagactttgcagcgtaccgcccctga

SEQ ID NO: 21 - protein, 740 aa, synthetic construct
MASPLTRFLSLNLLLLGESIILGSGEADIQMTQSPASLSTSLGETVTIQCQASEDIYSGLAWYQQKPGKSPQLLIYGASDLQDGVPSRFSGSGSGTQYSLKITSMQTEDEGVYFCQQGLTYPRTFGGGTKLELKGGGGSGGGGSGGGGSEVQLQQSGAELVRPGTSVKLSCKVSGDTITFYYMHFVKQRPGQGLEWIGRIDPEDESTKYSEKFKNKATLTADTSSNTAYLKLSSLTSEDTATYFCIYGGYYFDYWGQGVMVTVSSTTTKPVLRTPSPVHPTGTSQPQRPEDCRPRGSVKGTGLDFACDIYIWAPLAGICVALLLSLIITLICKRGRKKLLYIFKQPFMRPVQTTQEEDGCSCRFPEEEEGGCELRAKFSRSAETAANLQDPNQLYNELNLGRREEYDVLEKKRARDPEMGGKQQRRRNPQEGVYNALQKDKMAEAYSEIGTKGERRRGKGHDGLYQGLSTATKDTYDALHMQTLAPRGSGATNFSLLKQAGDVEENPGPMACLGLRRYKAQLQLPSRTWPFVALLTLLFIPVFSEAIQVTQPSVVLASSHGVASFPCEYSPSHNTDEVRVTVLRQTNDQMTEVCATTFTEKNTVGFLDYPFCSGTFNESRVNLTIQGLRAVDTGLYLCKVELMYPPPYFVGMGNGTQIYVIDPEPCPDSDFLLWILVAVSLGLFFYSFLVTAVSLSKMTNSRRNRLLQSDYMNMTPRRPGLTRKPYQPYAPARDFAAYRP

SEQ ID NO: 22 - DNA, 2220 bp, synthetic construct
  source 1..2220: mol_type = other DNA
atggccttaccagtgaccgccttgctcctgccgctggccttgctgctccacgccgccaggccggacatccagatgacacagactacatcctccctgtctgcctctctgggagacagagtcaccatcagttgcagggcaagtcaggacattagtaaatatttaaattggtatcagcagaaaccagatggaactgttaaactcctgatctaccatacatcaagattacactcaggagtcccatcaaggttcagtggcagtgggtctggaacagattattctctcaccattagcaacctggagcaagaagatattgccacttacttttgccaacagggtaatacgcttccgtacacgttcggaggggggaccaagctggagatcacaggtggcggtggctcgggcggtggtgggtcgggtggcggcggatctgaggtgaaactgcaggagtcaggacctggcctggtggcgccctcacagagcctgtccgtcacatgcactgtctcaggggtctcattacccgactatggtgtaagctggattcgccagcctccacgaaagggtctggagtggctgggagtaatatggggtagtgaaaccacatactataattcagctctcaaatccagactgaccatcatcaaggacaactccaagagccaagttttcttaaaaatgaacagtctgcaaactgatgacacagccatttactactgtgccaaacattattactacggtggtagctatgctatggactactggggccaaggaacctcagtcaccgtctcctcaaccacgacgccagcgccgcgaccaccaacaccggcgcccaccatcgcgtcgcagcccctgtccctgcgcccagaggcgtgccggccagcggcggggggcgcagtgcacacgagggggctggacttcgcctgtgatatctacatctgggcgcccttggccgggacttgtggggtccttctcctgtcactggttatcaccctttactgcaaacggggcagaaagaaactcctgtatatattcaaacaaccatttatgagaccagtacaaactactcaagaggaagatggctgtagctgccgatttccagaagaagaagaaggaggatgtgaactgagagtgaagttcagcaggagcgcagacgcccccgcgtacaagcagggccagaaccagctctataacgagctcaatctaggacgaagagaggagtacgatgttttggacaagagacgtggccgggaccctgagatggggggaaagccgagaaggaagaaccctcaggaaggcctgtacaatgaactgcagaaagataagatggcggaggcctacagtgagattgggatgaaaggcgagcgccggaggggcaaggggcacgatggcctttaccagggtctcagtacagccaccaaggacacctacgacgcccttcacatgcaggccctgccccctcgcggatctggcgccaccaatttcagcctgctgaaacaggctggcgacgtggaagagaaccctggacctatggcctgcctgggcttccagagacacaaggcccaactgaacctggccaccagaacatggccctgtactctgctgttcttcctgctgttcatccccgtgttctgcaaggccatgcatgtggctcagccagctgtggtgctggcctcttctagaggaatcgccagcttcgtgtgcgagtacgcctctcctggaaaggccactgaagtgcgcgtgaccgttctgagacaggccgatagccaagtgaccgaagtgtgcgccgccacctacatgatgggcaacgagctgaccttcctggacgacagcatctgtaccggcaccagcagcggcaatcaagtgaacctgaccatccagggcctgagagccatggataccggcctgtacatctgcaaggtggaactgatgtaccctcctccttactacctcggcatcggcaacggcacccagatctacgtgatcgaccctgagccttgtcctgacagcgactttctgctgtggattctggccgccgtgtccagcggcctgttcttctactcttttctgctgaccgctgtgtccctgagcaagatggtccgaagcaagcggagcagactgctgcacagcgactacatgaacatgacccctagacggcccggacctaccagaaagcactaccagccttacgctcctcctagagacttcgccgcctacagaagctga

SEQ ID NO: 23 - protein, 739 aa, synthetic construct
MALPVTALLLPLALLLHAARPDIQMTQTTSSLSASLGDRVTISCRASQDISKYLNWYQQKPDGTVKLLIYHTSRLHSGVPSRFSGSGSGTDYSLTISNLEQEDIATYFCQQGNTLPYTFGGGTKLEITGGGGSGGGGSGGGGSEVKLQESGPGLVAPSQSLSVTCTVSGVSLPDYGVSWIRQPPRKGLEWLGVIWGSETTYYNSALKSRLTIIKDNSKSQVFLKMNSLQTDDTAIYYCAKHYYYGGSYAMDYWGQGTSVTVSSTTTPAPRPPTPAPTIASQPLSLRPEACRPAAGGAVHTRGLDFACDIYIWAPLAGTCGVLLLSLVITLYCKRGRKKLLYIFKQPFMRPVQTTQEEDGCSCRFPEEEEGGCELRVKFSRSADAPAYKQGQNQLYNELNLGRREEYDVLDKRRGRDPEMGGKPRRKNPQEGLYNELQKDKMAEAYSEIGMKGERRRGKGHDGLYQGLSTATKDTYDALHMQALPPRGSGATNFSLLKQAGDVEENPGPMACLGFQRHKAQLNLATRTWPCTLLFFLLFIPVFCKAMHVAQPAVVLASSRGIASFVCEYASPGKATEVRVTVLRQADSQVTEVCAATYMMGNELTFLDDSICTGTSSGNQVNLTIQGLRAMDTGLYICKVELMYPPPYYLGIGNGTQIYVIDPEPCPDSDFLLWILAAVSSGLFFYSFLLTAVSLSKMVRSKRSRLLHSDYMNMTPRRPGPTRKHYQPYAPPRDFAAYRS